European Patent Application EP 4 592 677 A1, published July 30, 2025. Title: Method for Assisting Decision of Treatment Direction for Dogs with Skin Symptoms. Applicant: 日本全薬工業株式会社. The sequence listing filed with the application follows.

SEQUENCE LISTING (3 sequences)

SEQ ID NO: 1 - protein, 99 aa, Canis lupus familiaris
MIPLKMLLLVTLLLGASLQVTHAARGTNVGRECCLEYFKGAIPISRLTRWYKTSGECPKDAIVFVTVQGKSICSDPKDKRVKKAVRYLQRTWKGGPQES

SEQ ID NO: 2 - protein, 147 aa, Mus musculus
MGKCAAMGRLTSSFLLLIVPAYVLSQVTLKESGPGILQPSQTLSLTCSFSGFSLNTSGMGVGWIRQPSGKGLEWLAHIWWDDDKRYNPALKSRLTISKDTFNNQVFLNIASVDTADTATYYCARIYFGSSLAWFAYWGQGTLVTVSA

SEQ ID NO: 3 - protein, 144 aa, Mus musculus
MGTQDFLYQVLRMRCLAEFLGLLVLWIPGAIGDIVMTQATSSVFVTPGDSVSISCRSSKSLLHSNGNTYLYWFLQRPGQSPQLLIYRMSNLASGVPDRFSGSGSGTAFTLRISRVEAEDVGVYYCMQHLENPTFGAGTKLELKR